European Patent Application EP 4 549 571 A1, published May 7, 2025. Title: Mutant Nitrile Hydratase, Nucleic Acid Encoding the Mutant Nitrile Hydratase, Expression Vector and Transformant Containing the Nucleic Acid, Production Method for Muntant Nitrile Hydratase, and Production Method for Amide Compound. Applicant: MITSUI CHEMICALS, INC. The sequence listing filed with the application follows.

SEQUENCE LISTING (36 sequences)

SEQ ID NO: 1 - protein, 205 aa, Pseudonocardia thermophila
MTENILRKSDEEIQKEITARVKALESMLIEQGILTTSMIDRMAEIYENEVGPHLGAKVVVKAWTDPEFKKRLLADGTEACKELGIGGLQGEDMMWVENTDEVHHVVVCTLCSCYPWPVLGLPPNWFKEPQYRSRVVREPRQLLKEEFGFEVPPSKEIKVWDSSSEMRFVVLPQRPAGTDGWSEEELATLVTRESMIGVEPAKAVA

SEQ ID NO: 2 - protein, 233 aa, Pseudonocardia thermophila
MNGVYDVGGTDGLGPINRPADEPVFRAEWEKVAFAMFPATFRAGFMGLDEFRFGIEQMNPAEYLESPYYWHWIRTYIHHGVRTGKIDLEELERRTQYYRENPDAPLPEHEQKPELIEFVNQAVYGGLPASREVDRPPKFKEGDVVRFSTASPKGHARRARYVRGKTGTVVKHHGAYIYPDTAGNGLGECPEHLYTVRFTAQELWGPEGDPNSSVYYDCWEPYIELVDTKAAAA

SEQ ID NO: 3 - DNA, 618 bp, Pseudonocardia thermophila
  source 1..618: mol_type = genomic DNA
atgaccgagaacatcctgcgcaagtcggacgaggagatccagaaggagatcacggcgcgggtcaaggccctggagtcgatgctcatcgaacagggcatcctcaccacgtcgatgatcgaccggatggccgagatctacgagaacgaggtcggcccgcacctcggcgcgaaggtcgtcgtgaaggcctggaccgacccggagttcaagaagcgtctgctcgccgacggcaccgaggcctgcaaggagctcggcatcggcggcctgcagggcgaggacatgatgtgggtggagaacaccgacgaggtccaccacgtcgtcgtgtgcacgctctgctcctgctacccgtggccggtgctggggctgccgccgaactggttcaaggagccgcagtaccgctcccgcgtggtgcgtgagccccggcagctgctcaaggaggagttcggcttcgaggtcccgccgagcaaggagatcaaggtctgggactccagctccgagatgcgcttcgtcgtcctcccgcagcgccccgcgggcaccgacgggtggagcgaggaggagctcgccaccctcgtcacccgcgagtcgatgatcggcgtcgaaccggcgaaggcggtcgcgtga

SEQ ID NO: 4 - DNA, 702 bp, Pseudonocardia thermophila
  source 1..702: mol_type = genomic DNA
atgaacggcgtgtacgacgtcggcggcaccgatgggctgggcccgatcaaccggcccgcggacgaaccggtcttccgcgccgagtgggagaaggtcgcgttcgcgatgttcccggcgacgttccgggccggcttcatgggcctggacgagttccggttcggcatcgagcagatgaacccggccgagtacctcgagtcgccgtactactggcactggatccgcacctacatccaccacggcgtccgcaccggcaagatcgatctcgaggagctggagcgccgcacgcagtactaccgggagaaccccgacgccccgctgcccgagcacgagcagaagccggagttgatcgagttcgtcaaccaggccgtctacggcgggctgcccgcaagccgggaggtcgaccgaccgcccaagttcaaggagggcgacgtggtgcggttctccaccgcgagcccgaagggccacgcccggcgcgcgcggtacgtgcgcggcaagaccgggacggtggtcaagcaccacggcgcgtacatctacccggacaccgccggcaacggcctgggcgagtgccccgagcacctctacaccgtccgcttcacggcccaggagctgtgggggccggaaggggacccgaactccagcgtctactacgactgctgggagccctacatcgagctcgtcgacacgaaggcggccgcggcatga

SEQ ID NO: 5 - DNA, 33 bp, synthetic construct
  misc_feature 1..33: note = Primer
  source 1..33: mol_type = other DNA
acggtgcgggtcaagggcctggagtcgatgctc

SEQ ID NO: 6 - DNA, 33 bp, synthetic construct
  misc_feature 1..33: note = Primer
  source 1..33: mol_type = other DNA
gacgaggtccaccacatggtcgtgtgcacgctc

SEQ ID NO: 7 - DNA, 33 bp, synthetic construct
  misc_feature 1..33: note = Primer
  source 1..33: mol_type = other DNA
cgtgagccccggcagtgcctcaaggaggagttc

SEQ ID NO: 8 - DNA, 33 bp, synthetic construct
  misc_feature 1..33: note = Primer
  source 1..33: mol_type = other DNA
cggcagctgctcaaggacgagttcggcttcgag

SEQ ID NO: 9 - DNA, 33 bp, synthetic construct
  misc_feature 1..33: note = Primer
  source 1..33: mol_type = other DNA
ttcggcttcgaggtcgggccgagcaaggagatc

SEQ ID NO: 10 - DNA, 33 bp, synthetic construct
  misc_feature 1..33: note = Primer
  source 1..33: mol_type = other DNA
ggcttcgaggtcccgcgcagcaaggagatcaag

SEQ ID NO: 11 - DNA, 33 bp, synthetic construct
  misc_feature 1..33: note = Primer
  source 1..33: mol_type = other DNA
cccgcgggcaccgacgtgtggagcgaggaggag

SEQ ID NO: 12 - DNA, 33 bp, synthetic construct
  misc_feature 1..33: note = Primer
  source 1..33: mol_type = other DNA
ggcaagatcgatctcctcgagctggagcgccgc

SEQ ID NO: 13 - DNA, 33 bp, synthetic construct
  misc_feature 1..33: note = Primer
  source 1..33: mol_type = other DNA
gagttcgtcaaccagatagtctacggcgggctg

SEQ ID NO: 14 - DNA, 33 bp, synthetic construct
  misc_feature 1..33: note = Primer
  source 1..33: mol_type = other DNA
gtggtgcggttctcccaagcgagcccgaagggc

SEQ ID NO: 15 - DNA, 33 bp, synthetic construct
  misc_feature 1..33: note = Primer
  source 1..33: mol_type = other DNA
tccaccgcgagcccgcgtggccacgcccggcgc

SEQ ID NO: 16 - DNA, 33 bp, synthetic construct
  misc_feature 1..33: note = Primer
  source 1..33: mol_type = other DNA
aacggcctgggcgagtcccccgagcacctctac

SEQ ID NO: 17 - DNA, 33 bp, synthetic construct
  misc_feature 1..33: note = Primer
  source 1..33: mol_type = other DNA
gagctgtgggtgccggggggggacccgaactac

SEQ ID NO: 18 - DNA, 33 bp, synthetic construct
  misc_feature 1..33: note = Primer
  source 1..33: mol_type = other DNA
gacactaaggaggtctgggcatgaccgagaaca

SEQ ID NO: 19 - DNA, 33 bp, synthetic construct
  misc_feature 1..33: note = Primer
  source 1..33: mol_type = other DNA
actaaggaggtcgcgagatgaccgagaacatca

SEQ ID NO: 20 - DNA, 33 bp, synthetic construct
  misc_feature 1..33: note = Primer
  source 1..33: mol_type = other DNA
gaggaggagctcgccaaactcgtcactcgcgag

SEQ ID NO: 21 - DNA, 33 bp, synthetic construct
  misc_feature 1..33: note = Primer
  source 1..33: mol_type = other DNA
ttcatgggcgtggacgggttccggttcggcatc

SEQ ID NO: 22 - DNA, 33 bp, synthetic construct
  misc_feature 1..33: note = Primer
  source 1..33: mol_type = other DNA
cactggatccgcacctgcatccacaacggcgtc

SEQ ID NO: 23 - DNA, 33 bp, synthetic construct
  misc_feature 1..33: note = Primer
  source 1..33: mol_type = other DNA
gtgcgtgagccccggcgactgctcaaggaggag

SEQ ID NO: 24 - DNA, 33 bp, synthetic construct; identical to SEQ ID NO: 21
  misc_feature 1..33: note = Primer
  source 1..33: mol_type = other DNA

SEQ ID NO: 25 - DNA, 33 bp, synthetic construct; identical to SEQ ID NO: 6
  misc_feature 1..33: note = Primer
  source 1..33: mol_type = other DNA

SEQ ID NO: 26 - DNA, 33 bp, synthetic construct
  misc_feature 1..33: note = Primer
  source 1..33: mol_type = other DNA
ggttggagcgaggaggcactcgccaccctcgtc

SEQ ID NO: 27 - DNA, 33 bp, synthetic construct
  misc_feature 1..33: note = Primer
  source 1..33: mol_type = other DNA
gagggcgacgtggtgcagttctccaccgcgagc

SEQ ID NO: 28 - DNA, 33 bp, synthetic construct
  misc_feature 1..33: note = Primer
  source 1..33: mol_type = other DNA
cacgcccggcgcgcgcaatacgtgcgcggcaag

SEQ ID NO: 29 - DNA, 33 bp, synthetic construct
  misc_feature 1..33: note = Primer
  source 1..33: mol_type = other DNA
aagcaccacggcgcgtgcatctacccggacacc

SEQ ID NO: 30 - DNA, 33 bp, synthetic construct
  misc_feature 1..33: note = Primer
  source 1..33: mol_type = other DNA
cacaacggcgtccgccacggcaagatcgatctc

SEQ ID NO: 31 - DNA, 33 bp, synthetic construct
  misc_feature 1..33: note = Primer
  source 1..33: mol_type = other DNA
cccgcaagccgggagcgcgaccgaccgcccaag

SEQ ID NO: 32 - DNA, 33 bp, synthetic construct
  misc_feature 1..33: note = Primer
  source 1..33: mol_type = other DNA
accggcaagatcgatcgggaggagctggagcgc

SEQ ID NO: 33 - DNA, 17 bp, synthetic construct
  misc_feature 1..17: note = Primer
  source 1..17: mol_type = other DNA
gttttcccagtcacgac

SEQ ID NO: 34 - DNA, 20 bp, synthetic construct
  misc_feature 1..20: note = Primer
  source 1..20: mol_type = other DNA
ggccagtgcctagcttacat

SEQ ID NO: 35 - DNA, 17 bp, synthetic construct
  misc_feature 1..17: note = Primer
  source 1..17: mol_type = other DNA
caggaaacagctatgac

SEQ ID NO: 36 - protein, 144 aa, synthetic construct
  REGION 1..144: note = Pseudonocardia thermophila
MSAEAKVRLKHCPTAEDRAAADALLAQLPGGDRALDRGFDEPWQLRAFALAVAACRAGRFEWKQLQQALISSIGEWERTHDLDDPSWSYYEHFVAALESVLGEEGIVEPEALDERTAEVLANPPNKDHHGPHLEPVAVHPAVRS